European Patent Application EP 4 606 904 A1, published August 27, 2025. Title: 阿糖类核苷一锅法生物合成的方法及组合物. Applicant: 凯莱英生命科学技术（天津）有限公司. The sequence listing filed with the application follows.

SEQUENCE LISTING (6 sequences)

SEQ ID NO: 1 - protein, 344 aa, Trypanosoma cruzi
MSKATHTHGLMKDPDLPVTADGVTYHLNCKSDQLADRILLVGDPGRVDTVAACFDAGSVRFRSENREIFIATGTYKGTPVSVLSTGMGTDNVEIVINEIHLLKEYDFERCSWRPRVGDADVPPGAKVFDPSSVKMIRVGTCGSPFPDMPLAALAITRHVIGMDNTCLYYKVKEQMQKSKDLQEVQRVVKEQTSLGAIDVYATKAHPAITNGIVAACKAFNDNLPAGATEQLYVVGATATASGFYACQGRAVGRFREHLLVPKLVEELSKVQFDVSEGKEIVANIEMETSAVCFLSHLLGYQAGSMCVVVAKRAGAEHLFTTSEQSGQALKNAIQIALEAIVAVG

SEQ ID NO: 2 - protein, 423 aa, Thermus thermophiles
MNPVAFIREKREGKKHRREDLEAFLLGYLRDEVPDYQVSAWLMAAFLRGLDPEETLWLTETMARSGKVLDLSGLPHPVDKHSSGGVGDKVSLVVGPILAASGCTFAKMSGRGLAHTGGTIDKLESVPGWRGEMTEAEFLERARRVGLVIAAQSPDLAPLDGKLYALRDVTATVESVPLIASSIMSKKLAAGARSIVLDVKVGRGAFMKTLEEARLLAKTMVAIGQGAGRRVRALLTSMEAPLGRAVGNAIEVREAIEALKGEGPGDLLEVALALAEEALRLEGLDPALARKALEGGAALEKFRAFLEAQGGDPRAVEDFSLLPLAEEHPLRAEREGVVREVDAYKVGLAVLALGGGRKRKGEPIDHGVGVYLLKKPGDRVERGEALALVYHRRRGLEEALGHLREAYALGEEAHPAPLVLEAI

SEQ ID NO: 3 - protein, 234 aa, Geobacillus stearothermophilus
MSVHIGAKEHEIADKILLPGDPLRAKYIAETFLEGATCYNQVRGMLGFTGTYKGHRISVQGTGMGVPSISIYITELMQSYNVQTLIRVGTCGAIQKDVKVRDVILAMTSSTDSQMNRMTFGGIDYAPTANFDLLKTAYEIGKEKGLQLKVGSVFTADMFYNENAQFEKLARYGVLAVEMETTALYTLAAKFGRKALSVLTVSDHILTGEETTAEERQTTFNEMIEVALETAIRQ

SEQ ID NO: 4 - DNA, 1035 bp, synthetic construct
  source 1..1035: mol_type = other DNA; note; note (original language) = 编码UP的DNA序列
atgagcaaagcgacccatacccacggcctgatgaaagatccggatctgccggtgacggcggatggcgttacctatcatctgaactgcaaaagcgatcagctggcggatcgcattctgctggtgggcgatccgggtcgcgttgataccgtagcggcatgttttgatgcgggcagcgttcgctttcgcagcgaaaaccgcgaaatttttattgcgaccggcacctataaaggcaccccggtgtcagtgctgagcaccggtatgggtactgataatgtggaaattgtgattaacgagattcacctgctgaaggagtatgacttcgagcgctgcagctggcgcccgcgtgttggtgatgcggatgttcctcctggtgcgaaagtgtttgatccgagcagcgtgaaaatgattcgcgtgggcacctgcggcagcccgtttcctgatatgcctctggcggcgctggcgattacccgccatgttattggcatggataacacctgcctgtattataaagtgaaagagcagatgcagaagagcaaggatctgcaggaagtgcagcgcgtggtgaaagaacagaccagcctgggcgcgattgatgtgtatgcgaccaaagcgcatccggcgattaccaacggcattgtggcggcgtgtaaagcgtttaacgataacctgccggcgggcgcgactgaacaattatatgttgttggcgcgaccgcgaccgcgagcggtttttatgcgtgtcaaggtcgcgcggtgggccgctttcgtgaacatttactggttccgaaactggtggaagaactgagcaaagtgcagtttgatgtgagcgaaggcaaagaaattgtggcgaacattgaaatggaaaccagcgcggtgtgctttctgagccatctgctgggctatcaggcgggctcaatgtgcgttgttgttgcgaaacgcgcgggcgcggaacatctgtttaccaccagcgaacagagcggccaggcgctgaaaaacgcgattcagattgcgctggaagcgattgtggcggtgggctaa

SEQ ID NO: 5 - DNA, 1272 bp, synthetic construct
  source 1..1272: mol_type = other DNA; note; note (original language) = 编码PyNP的DNA序列
atgaacccggtggcgtttattcgcgaaaaacgcgaaggcaagaaacatcgccgcgaggatctggaagcgtttctgctgggctatctgcgcgatgaagtgccggattatcaggtgagcgcgtggctgatggcggcgtttttacgcggcttagatccggaagaaaccctgtggctgaccgaaacgatggcccgcagcggtaaagtgctggatctgagcggtctgccgcatccggttgataaacatagcagcggcggcgtgggcgataaagtgagcttagtggtgggcccgattctggcggcgagcggttgtacctttgcgaaaatgtcgggccgcggcctggcgcataccggtggtaccattgataaactggaaagcgtgccgggctggcgcggcgaaatgaccgaagcagaatttctggaacgcgcccgtcgcgttggtctggttattgcggcgcaaagcccggatttagcgccgttagatggcaaactgtatgcgctgcgcgatgtgaccgcgaccgttgaatcagttccgctgattgcgagcagcattatgagcaagaaactggcggcgggcgcccgtagcattgtgttagatgttaaagtgggccgcggcgcgtttatgaaaaccctggaagaagcgcgtctgctggcgaaaacgatggtggcgattggccagggcgcgggccgtcgtgttcgtgcgttattaaccagcatggaagcgcctctgggtcgtgcggttggcaatgcgattgaagtgcgtgaagcgattgaagcgctgaaaggcgaaggcccgggcgatttattagaagtggcgctggcgttagcggaagaagcgctgcgtttagaaggcttagatccggcgctggcgcgtaaagcgttagaaggtggcgcggcgctggaaaaatttcgcgcgtttctggaagcgcagggcggcgatccgcgtgcagttgaagattttagcctgctgccgctggcggaagaacatccgttacgtgcggaacgcgaaggcgtggttcgcgaagttgatgcgtataaagtgggcctggcggtgctggcgttaggcggtggtcgtaaacgtaaaggtgaaccgattgatcatggcgtgggcgtgtatctgctgaagaaaccgggcgatcgcgtggaacgcggcgaagcgttagcgttagtgtatcatcgccgccgcggcttagaagaagcgctgggtcatttacgcgaagcgtatgcgctgggcgaagaagcgcatccggcgcctctggttttagaagcgatttaa

SEQ ID NO: 6 - DNA, 705 bp, synthetic construct
  source 1..705: mol_type = other DNA; note; note (original language) = 编码PNP的DNA序列
atgagcgtgcatattggcgcgaaagaacatgaaattgcggataaaattctgctgccgggcgatccgttacgcgcgaaatatattgcggaaacctttctggaaggcgcgacctgctataaccaggtgcgcggcatgctgggctttaccggcacctataaaggccatcgcattagcgtgcagggcaccggcatgggcgttcctagcatttcaatttatattaccgaactgatgcagagctataacgtgcagaccctgattcgcgtgggcacctgcggtgcgattcaaaaagatgtgaaagtgcgcgatgtgattctggcgatgaccagcagcaccgatagccagatgaaccgcatgacctttggcggcattgattatgcgccgaccgcgaactttgatctgctgaaaaccgcgtatgaaattggcaaagaaaaaggcctgcagctgaaagtgggcagcgtgtttaccgcggatatgttttataacgaaaacgcgcagtttgagaaactggcccgctatggcgtgctggcggttgaaatggaaaccaccgcgctgtataccctggcggcgaaatttggccgcaaagcgctgagcgtgctgaccgtgagcgatcatattctgaccggcgaagaaaccaccgcggaagaacgccagaccacctttaacgaaatgattgaagtggcgctggaaaccgcgattcgccagtaa